European Patent Specification EP 4 022 090 B1, published March 18, 2026. Title: REAGENTS, KITS AND METHODS FOR ASSESSING AND REDUCING RISK. Applicant: Hill's Pet Nutrition, Inc. The sequence listing filed with the application follows.

SEQUENCE LISTING (2 sequences)

SEQ ID NO: 1 - DNA, 200 bp, Canis familiaris
tcaaattcccattcttggcaacaagcacccaccacccctctgcctgacacattctgctctcttccttcgttcccttcttgcatgaccgccccacacaccgycttcattgagcagatataattgccccttctttaaacctcaatccagggacccctgggtggttcagtggtgagtgtctgcctttggctcagggtgtaatc

SEQ ID NO: 2 - DNA, 201 bp, Canis familiaris
ccaccttttcttccttttgttcagttattttaattctgtcttcatcaaagcccatcccaagaataagggagtatattgcagttttgcgattaacgcgagcrctagaagaaacacttctatgtcagcaaaatgtccccgtgttctgggagagaactttgaaggaggacgggggaagtgcagcagtgtttactgacagtccag